European Patent Application EP 4 534 645 A1, published April 9, 2025. Title: MICROZYME, MICROZYME POWDER AND APPLICATION THEREOF IN PASTA PROCESSING. Applicant: SHENZHEN TAISU BIOTECHNOLOGY CO., LTD. Application US. The sequence listing filed with the application follows.

SEQUENCE LISTING (1 sequence)

SEQ ID NO: 1 - DNA, 1793 bp, Monosporozyma servazzii
  source 1..1793: chromosome = 12 704328 to 706120 Sequence ID: CP138606.1; mol_type = other DNA; strain = YE05
atctggttgatcctgccagtagtcatatgcttgtctcaaagattaagccatgcatgtctaagtataagcaatttatacagtgaaactgcgaatggctcattaaatcagttatcgtttatttgatagttcctttactacatggtataactgtggtaattctagagctaatacatgcttaaaatcccgaccttttggaagggatgtatttattagataaaaaatcaatgtcttcggactctttgatgattcataataacttttcgaatcgcatggccttgtgccggcgatggttcattcaaatttctgccctatcaactttcgatggtaggatagtggcctaccatggtttcaacgggtaacggggaataagggttcgattccggagagggagcctgagaaacggctaccacatccaaggaaggcagcaggcgcgcaaattacccaatcctaatacagggaggtagtgacaataaataacgatacagggccctttcgggtcttgtaattggaatgagtacaatgtaaataccttaacgaggaacaattggagggcaagtctggtgccagcagccgcggtaattccagctccaatagcgtatattaaagttgttgcagttaaaagctcgtagttgaactttgggcctggttggccggtctggctttttgccacgtactggaatgcaaccgggcctttccttctggctaaccttaggctccttgtgggtctttggcgaaccaggacttttactttgaaaaaattagagtgttcaaagcaggcgtattgctcgaatatattagcatggaataatggaataggacgtttggttctattttgttggtttctaggaccatcgtaatgattaatagggacggtcgggggcatcagtattcaattgtcagaggtgaaattcttggatttattgaagactaactactgcgaaagcatttgccaaggacgttttcattaatcaagaacgaaagttaggggatcgaagatgatcagataccgtcgtagtcttaaccataaactatgccgactagggatcgggtggtgtttttaatgacccactcggcaccttacgagaaatcaaagtctttgggttctggagtatggtcgcaaggctgaaacttaaaggaattgacggaagggcaccaccaggagtggagcctgcggcttaatttgactcaacacggggaaactcaccaggtccagacacaataaggattgacagattgagagctctttcttgattttgtgggtggtggtgcatggccgttcttagttggtggagtgatttgtctgcttaattgcgataacgaacgagaccttaacctactaaatagtggtgctagcatttgctggttcttccacttcttagagggactatcgatttcaagtcgatggaagtttgaggcaataacaggtctgtgatgcccttagacgttctgggccgcacgcgcgctacactgacggagccagcgagtctaacctaggccgagaggtcctggtaatcttgtgaaactccgtcgtgctggggatagagctttgtaatttttgctcttcaacgaggaattcctagtaagcgcaagtcatcagcttgcgttgattacgtcctgccctttgtacacaccgcccgtcgctagtaccgattgaatggcttagtgaggcctcaggatctgctagagaaggggcaactccatctcagagcggaaaatctggtcaaacttggtcatttagaggaactaaaagtcgtaacaaggtttccgtaggtgaacctgcggaaggatcatta